European Patent Application EP 4 582 557 A1, published July 9, 2025. Title: Rapid Sterility Test. Applicant: 島津ダイアグノスティクス株式会社. The sequence listing filed with the application follows.

SEQUENCE LISTING (60 sequences)

SEQ ID NO: 1 - DNA, 13 bp, synthetic construct
  source 1..13: mol_type = other DNA
ccagcagccgcgg

SEQ ID NO: 2 - DNA, 16 bp, synthetic construct
  source 1..16: mol_type = other DNA
gtgccagcagccgcgg

SEQ ID NO: 3 - DNA, 19 bp, synthetic construct
  source 1..19: mol_type = other DNA
gtgccagcagccgcggtaa

SEQ ID NO: 4-5 - skipped (2 entries)

SEQ ID NO: 6 - DNA, 10 bp, synthetic construct
  source 1..10: mol_type = other DNA
gctcgttgcg

SEQ ID NO: 7 - DNA, 19 bp, synthetic construct
  source 1..19: mol_type = other DNA
gctcgttgcgggacttaac

SEQ ID NO: 8 - DNA, 20 bp, synthetic construct
  source 1..20: mol_type = other DNA
cgctcgttacgggacttaac

SEQ ID NO: 9 - DNA, 20 bp, synthetic construct
  source 1..20: mol_type = other DNA
cgctcgttgcaggacttaac

SEQ ID NO: 10 - DNA, 16 bp, synthetic construct
  source 1..16: mol_type = other DNA
gggttgcgctcgttgc

SEQ ID NO: 11 - DNA, 17 bp, synthetic construct
  source 1..17: mol_type = other DNA
gggttgcgctcgttgcg

SEQ ID NO: 12 - DNA, 25 bp, synthetic construct
  source 1..25: mol_type = other DNA
gggttgcgctcgttgcgggacttaa

SEQ ID NO: 13 - DNA, 26 bp, synthetic construct
  source 1..26: mol_type = other DNA
gggttgcgctcgttgcgggacttaac

SEQ ID NO: 14 - DNA, 27 bp, synthetic construct
  source 1..27: mol_type = other DNA
gggttgcgctcgttgcgggacttaacc

SEQ ID NO: 15 - DNA, 17 bp, synthetic construct
  source 1..17: mol_type = other DNA
ttgcgctcgttgcggga

SEQ ID NO: 16 - DNA, 17 bp, synthetic construct
  source 1..17: mol_type = other DNA
tgcgctcgttgcgggac

SEQ ID NO: 17 - DNA, 19 bp, synthetic construct
  source 1..19: mol_type = other DNA
ctcgttgcgggacttaacc

SEQ ID NO: 18 - DNA, 12 bp, synthetic construct
  source 1..12: mol_type = other DNA
gagctgacgaca

SEQ ID NO: 19 - DNA, 15 bp, synthetic construct
  source 1..15: mol_type = other DNA
cacgagctgacgaca

SEQ ID NO: 20 - DNA, 16 bp, synthetic construct
  source 1..16: mol_type = other DNA
cacgagctgacgacaa

SEQ ID NO: 21 - DNA, 23 bp, synthetic construct
  source 1..23: mol_type = other DNA
cacgagctgacgacaaccatgca

SEQ ID NO: 22 - DNA, 23 bp, synthetic construct
  source 1..23: mol_type = other DNA
cacgagctgacgacagccatgca

SEQ ID NO: 23 - DNA, 25 bp, synthetic construct
  source 1..25: mol_type = other DNA
catctcacgacacgagctgacgaca

SEQ ID NO: 24 - DNA, 39 bp, synthetic construct
  source 1..39: mol_type = other DNA
catctcacgacacgagctgacgacaaccatgcaccacct

SEQ ID NO: 25 - DNA, 20 bp, synthetic construct
  source 1..20: mol_type = other DNA
cacgacacgagctgacgaca

SEQ ID NO: 26 - DNA, 25 bp, synthetic construct
  source 1..25: mol_type = other DNA
agctgacgacaaccatgcaccacct

SEQ ID NO: 27 - skipped

SEQ ID NO: 28 - DNA, 14 bp, synthetic construct
  source 1..14: mol_type = other DNA
cacgacacgagctg

SEQ ID NO: 29 - DNA, 19 bp, synthetic construct
  source 1..19: mol_type = other DNA
catctcacgacacgagctg

SEQ ID NO: 30-31 - skipped (2 entries)

SEQ ID NO: 32 - DNA, 19 bp, synthetic construct
  source 1..19: mol_type = other DNA
cgacaaccatgcaccacct

SEQ ID NO: 33 - DNA, 11 bp, synthetic construct
  source 1..11: mol_type = other DNA
gaaactcacca

SEQ ID NO: 34 - DNA, 14 bp, synthetic construct
  source 1..14: mol_type = other DNA
gaaactcaccaggt

SEQ ID NO: 35 - DNA, 16 bp, synthetic construct
  source 1..16: mol_type = other DNA
gaaactcaccaggtcc

SEQ ID NO: 36 - DNA, 17 bp, synthetic construct
  source 1..17: mol_type = other DNA
gaaactcaccaggtcca

SEQ ID NO: 37 - DNA, 19 bp, synthetic construct
  source 1..19: mol_type = other DNA
gggaaactcaccaggtcca

SEQ ID NO: 38 - DNA, 21 bp, synthetic construct
  source 1..21: mol_type = other DNA
gaaactcaccaggtccagaca

SEQ ID NO: 39 - DNA, 23 bp, synthetic construct
  source 1..23: mol_type = other DNA
gggaaactcaccaggtccagaca

SEQ ID NO: 40 - DNA, 22 bp, synthetic construct
  source 1..22: mol_type = other DNA
gggaaactcaccaggtccagac

SEQ ID NO: 41 - DNA, 21 bp, synthetic construct
  source 1..21: mol_type = other DNA
gggaaactcaccaggtccaga

SEQ ID NO: 42 - DNA, 20 bp, synthetic construct
  source 1..20: mol_type = other DNA
gggaaactcaccaggtccag

SEQ ID NO: 43 - DNA, 18 bp, synthetic construct
  source 1..18: mol_type = other DNA
gggaaactcaccaggtcc

SEQ ID NO: 44 - DNA, 17 bp, synthetic construct
  source 1..17: mol_type = other DNA
gggaaactcaccaggtc

SEQ ID NO: 45 - DNA, 16 bp, synthetic construct
  source 1..16: mol_type = other DNA
acggggaaactcacca

SEQ ID NO: 46 - DNA, 19 bp, synthetic construct
  source 1..19: mol_type = other DNA
acggggaaactcaccaggt

SEQ ID NO: 47 - DNA, 19 bp, synthetic construct
  source 1..19: mol_type = other DNA
aacacggggaaactcacca

SEQ ID NO: 48 - DNA, 37 bp, synthetic construct
  source 1..37: mol_type = other DNA
ttaatttgactcaacacggggaaactcaccaggtcca

SEQ ID NO: 49 - DNA, 19 bp, synthetic construct
  source 1..19: mol_type = other DNA
ttgactcaacacggggaaa

SEQ ID NO: 50 - DNA, 19 bp, synthetic construct
  source 1..19: mol_type = other DNA
aatttgactcaacacgggg

SEQ ID NO: 51 - DNA, 17 bp, synthetic construct
  source 1..17: mol_type = other DNA
gtacaaagggcagggac

SEQ ID NO: 52 - DNA, 21 bp, synthetic construct
  source 1..21: mol_type = other DNA
tgtgtacaaagggcagggacg

SEQ ID NO: 53 - DNA, 18 bp, synthetic construct
  source 1..18: mol_type = other DNA
gtacaaagggcagggacg

SEQ ID NO: 54 - DNA, 28 bp, synthetic construct
  source 1..28: mol_type = other DNA
cgggcggtgtgtacaaagggcagggacg

SEQ ID NO: 55 - DNA, 36 bp, synthetic construct
  source 1..36: mol_type = other DNA
agtagcgacgggcggtgtgtacaaagggcagggacg

SEQ ID NO: 56 - DNA, 17 bp, synthetic construct
  source 1..17: mol_type = other DNA
agaacggccatgcacca

SEQ ID NO: 57 - DNA, 20 bp, synthetic construct
  source 1..20: mol_type = other DNA
ctaagaacggccatgcacca

SEQ ID NO: 58 - DNA, 23 bp, synthetic construct
  source 1..23: mol_type = other DNA
ctaagaacggccatgcaccacca

SEQ ID NO: 59 - DNA, 495 bp, Staphylococcus aureus
  source 1..495: mol_type = genomic DNA
gtgccagcagccgcggtaatacgtaggtggcaagcgttatccggaattattgggcgtaaagcgcgcgtaggcggttttttaagtctgatgtgaaagcccacggctcaaccgtggagggtcattggaaactggaaaacttgagtgcagaagaggaaagtggaattccatgtgtagcggtgaaatgcgcagagatatggaggaacaccagtggcgaaggcgactttctggtctgtaactgacgctgatgtgcgaaagcgtggggatcaaacaggattagataccctggtagtccacgccgtaaacgatgagtgctaaacccgcacaagcggtggagcatgtggtttaattcgaagcaacgcgaagaaccttaccaaatcttgacatcctttgacaactctagagatagagcttccccttcgggggacaaagtgacaggtggtgcatggttgtcgtcagctcgtgtcgtgagatgttgggttaagtcccgcaacgagc

SEQ ID NO: 60 - DNA, 338 bp, Candida albicans
  source 1..338: mol_type = genomic DNA
gggaaactcaccaggtccagacacaataaggattgacagattgagagctctttcttgattttgtgggtggtggtgcatggccgttcttagttggtggagtgatttgtctgcttaattgcgataacgaacgagaccttaacctgctaaatagccaggcccgctttggcgggtcgccggcttcttagagggactatcggctcaagccgatggaagtttgaggcaataacaggtctgtgatgcccttagatgttctgggccgcacgcgcgctacactgacagagccaacgagttcatttccttagccgaaaggtttgttacgtccctgccctttgtacaca